European Patent Application EP 4 245 855 A1, published September 20, 2023. Title: anti-TSPAN8-anti-CD3 bispecific antibody and anti-TSPAN8 antibody. Applicant: Astellas Pharma Inc. National Cancer Center. The sequence listing filed with the application follows.

SEQUENCE LISTING (43 sequences)

SEQ ID NO: 1 - DNA, 807 bp, Artificial Sequence
  human TSPAN8-Myc-DDK
  CDS (1)..(807)
atggcaggtgtgagtgcctgtataaaatattctatgtttaccttcaacttcttgttctggctatgtggtatcttgatcctagcattagcaatatgggtacgaataagcaatgactctcaagcaatttttggttctgaagatgtaggctctagctcctacgttgctgtggacatattgattgctgtaggtgccatcatcatgattctgggcttcctggcatgctgcggtgctataaaagaaagtcgctgcatgcttctgttgtttttcataggcttgcttctgatcctgctcctgcaggtggcgacaggtatcctaggagctgttttcaaatctaagtctgatcgcattgtgaatgaaactctctatgaaaacacaaagcttttgagcgccacaggggaaagtgaaaaacaattccaggaagccataattgtgtttcaagaagagtttaaatgctgcggtttggtcaatggagctgctgattggggaaataattttcaacactatcctgaattatgtgcctgtctagataagcagagaccatgccaaagctataatggaaaacaagtttacaaagagacctgtatttctttcataaaagacttcttggcaaaaaatttgattatagttattggaatagcatttggactggcagttattgagatactgggtttggtgttttctatggtcctgtattgccagatcgggaacaaaacgcgtacgcggccgctcgagcagaaactcatctcagaagaggatctggcagcaaatgatatcctggattacaaggatgacgacgataaggtttaa

SEQ ID NO: 2 - protein, 268 aa, Artificial Sequence
  Synthetic Construct
MAGVSACIKYSMFTFNFLFWLCGILILALAIWVRISNDSQAIFGSEDVGSSSYVAVDILIAVGAIIMILGFLACCGAIKESRCMLLLFFIGLLLILLLQVATGILGAVFKSKSDRIVNETLYENTKLLSATGESEKQFQEAIIVFQEEFKCCGLVNGAADWGNNFQHYPELCACLDKQRPCQSYNGKQVYKETCISFIKDFLAKNLIIVIGIAFGLAVIEILGLVFSMVLYCQIGNKTRTRPLEQKLISEEDLAANDILDYKDDDDKV

SEQ ID NO: 3 - DNA, 1356 bp, Artificial Sequence
  16B11.1_HC
  CDS (1)..(1356)
caggttcagctggttgaatctggcggcggagttgttcagcctggcggatctctgagactgtcttgtgccgcctccggcttcaccttctcctcttacggaatgcactgggtccgacaggcccctggcaaaggattggaatgggtcgccgtgatttggtacgacggccggaacaagtactacgccgactccgtgaagggcagattcaccatctctcgggacaactccaagaacaccctgtacctgcagatgaactccctgagagccgaggacaccgccgtgtactactgcaccagagatcactccggctccggcagctactacatcgattattggggccagggcaccctggtcaccgtgtcctctgcttctaccaagggacccagcgtgttccctctggctccttccagcaagtctacctctggcggaacagctgctctgggctgcctggtcaaggactactttcctgagcctgtgaccgtgtcttggaactctggcgctctgacatctggcgtgcacacctttccagctgtgctgcagtcctccggcctgtactctctgtcctctgtcgtgaccgtgccttccagctctctgggaacccagacctacatctgcaatgtgaaccacaagccttccaacaccaaggtggacaagaaggtggaacccaagtcctgcgacaagacccacacctgtcctccatgtcctgctccagaactgctcggcggtccctccgttttcctgtttccacctaagcctaaggacaccctgatgatctctcggacccctgaagtgacatgcgtggtggtggatgtgtcccacgaggatcccgaagtgaagttcaattggtacgtggacggcgtggaagtgcacaacgccaagaccaagcctagagaggaacagtacaactccacctacagagtggtgtccgtgctgaccgtgctgcaccaggattggctgaacggcaaagagtacaagtgcaaggtgtccaacaaggccctgcctgctcctatcgaaaagaccatctccaaggctaagggccagcctcgggaacctcaggtttacacactgcctccatctcgggacgagctgaccaagaatcaggtgtccctgacctgcctcgtgaagggcttctacccttctgatatcgccgtggaatgggagtccaacggccagcctgagaacaactacaagacaacccctcctgtgctggactccgacggctcattcttcctgtactccaagctgacagtggataagtcccggtggcagcagggcaacgtgttctcttgttctgtgatgcacgaggccctgcacaaccactacacccagaagagtctgtctctgtcccctggcaagtga

SEQ ID NO: 4 - protein, 451 aa, Artificial Sequence
  Synthetic Construct
QVQLVESGGGVVQPGGSLRLSCAASGFTFSSYGMHWVRQAPGKGLEWVAVIWYDGRNKYYADSVKGRFTISRDNSKNTLYLQMNSLRAEDTAVYYCTRDHSGSGSYYIDYWGQGTLVTVSSASTKGPSVFPLAPSSKSTSGGTAALGCLVKDYFPEPVTVSWNSGALTSGVHTFPAVLQSSGLYSLSSVVTVPSSSLGTQTYICNVNHKPSNTKVDKKVEPKSCDKTHTCPPCPAPELLGGPSVFLFPPKPKDTLMISRTPEVTCVVVDVSHEDPEVKFNWYVDGVEVHNAKTKPREEQYNSTYRVVSVLTVLHQDWLNGKEYKCKVSNKALPAPIEKTISKAKGQPREPQVYTLPPSRDELTKNQVSLTCLVKGFYPSDIAVEWESNGQPENNYKTTPPVLDSDGSFFLYSKLTVDKSRWQQGNVFSCSVMHEALHNHYTQKSLSLSPGK

SEQ ID NO: 5 - DNA, 1356 bp, Artificial Sequence
  16B11.1_HC_H
  CDS (1)..(1356)
caggttcagctggttgaatctggcggcggagttgttcagcctggcggatctctgagactgtcttgtgccgcctccggcttcaccttctcctcttacggaatgcactgggtccgacaggcccctggcaaaggattggaatgggtcgccgtgatttggtacgacggccggaacaagtactacgccgactccgtgaagggcagattcaccatctctcgggacaactccaagaacaccctgtacctgcagatgaactccctgagagccgaggacaccgccgtgtactactgcaccagagatcactccggctccggcagctactacatcgattattggggccagggcaccctggtcaccgtgtcctctgcttctaccaagggacccagcgtgttccctctggctccttccagcaagtctacctctggcggaacagctgctctgggctgcctggtcaaggactactttcctgagcctgtgaccgtgtcttggaactctggcgctctgacatctggcgtgcacacctttccagctgtgctgcagtcctccggcctgtactctctgtcctctgtcgtgaccgtgccttccagctctctgggaacccagacctacatctgcaatgtgaaccacaagccttccaacaccaaggtggacaagaaggtggaacccaagtcctgcgacaagacccacacctgtcctccatgtcctgctccagaagctgctggcggcccttccgtgtttctgttccctccaaagcctaaggacaccctgatgatctctcggacccctgaagtgacctgcgtggtggtggatgtgtctcacgaggatcccgaagtgaagttcaattggtacgtggacggcgtggaagtgcacaacgccaagaccaagcctagagaggaacagtacggctccacctacagagtggtgtccgtgctgaccgtgctgcaccaggattggctgaacggcaaagagtacaagtgcaaggtgtccaacaaggccctgcctgctcctatcgaaaagaccatctccaaggccaagggccagcctagggaaccccaggtttacaccttgcctccatctcgggacgagctgaccaagaaccaggtgtccctgtcttgcgctgtgaagggcttctacccctccgatatcgccgtggaatgggagtctaatggccagcctgagaacaactacaagacaacccctcctgtgctggactccgacggctcattcttcctggtgtccaagctgacagtggacaagtccagatggcagcagggcaacgtgttctcctgcagcgtgatgcacgaggccctgcacaatcactacacccagaagtctctgtctctgagccccggcaaatga

SEQ ID NO: 6 - protein, 451 aa, Artificial Sequence
  Synthetic Construct
QVQLVESGGGVVQPGGSLRLSCAASGFTFSSYGMHWVRQAPGKGLEWVAVIWYDGRNKYYADSVKGRFTISRDNSKNTLYLQMNSLRAEDTAVYYCTRDHSGSGSYYIDYWGQGTLVTVSSASTKGPSVFPLAPSSKSTSGGTAALGCLVKDYFPEPVTVSWNSGALTSGVHTFPAVLQSSGLYSLSSVVTVPSSSLGTQTYICNVNHKPSNTKVDKKVEPKSCDKTHTCPPCPAPEAAGGPSVFLFPPKPKDTLMISRTPEVTCVVVDVSHEDPEVKFNWYVDGVEVHNAKTKPREEQYGSTYRVVSVLTVLHQDWLNGKEYKCKVSNKALPAPIEKTISKAKGQPREPQVYTLPPSRDELTKNQVSLSCAVKGFYPSDIAVEWESNGQPENNYKTTPPVLDSDGSFFLVSKLTVDKSRWQQGNVFSCSVMHEALHNHYTQKSLSLSPGK

SEQ ID NO: 7 - DNA, 642 bp, Artificial Sequence
  16B11.1_LC
  CDS (1)..(642)
gagattgccatgacacagtctcccgccacactgtctgttagccctggcgagagagctaccctgtcctgtagagcctctcagtccgtgtcctctaacctggcctggtatcagcagaagcctggacaggctccccggctgttgatctatggcgcttctaccagagctaccggcctgcctgctagattctccggctctggatctggcaccgagtttaccctgaccatctccagcctgcagtccgaggatttcgccgtgtactactgccagcagtacaacaacttctggaccttcggccagggcaccaaggtggaaatcaagagaaccgtggccgctccttccgtgttcatcttcccaccttccgacgagcagctgaagtccggcacagcttctgtcgtgtgcctgctgaacaacttttaccctcgggaagccaaggtgcagtggaaggtggacaatgccctgcagagcggcaactcccaagagtctgtgaccgagcaggactccaaggacagcacctacagcctgtcctccacactgaccctgtccaaggccgactacgagaagcacaaggtgtacgcctgcgaagtgacccatcagggcctgtctagccctgtgaccaagtctttcaaccggggcgagtgctga

SEQ ID NO: 8 - protein, 213 aa, Artificial Sequence
  Synthetic Construct
EIAMTQSPATLSVSPGERATLSCRASQSVSSNLAWYQQKPGQAPRLLIYGASTRATGLPARFSGSGSGTEFTLTISSLQSEDFAVYYCQQYNNFWTFGQGTKVEIKRTVAAPSVFIFPPSDEQLKSGTASVVCLLNNFYPREAKVQWKVDNALQSGNSQESVTEQDSKDSTYSLSSTLTLSKADYEKHKVYACEVTHQGLSSPVTKSFNRGEC

SEQ ID NO: 9 - DNA, 1356 bp, Artificial Sequence
  16B12.1_HC
  CDS (1)..(1356)
caggttcagctggttgaatctggcggcggagttgttcagcctggcggatctctgagactgtcttgtgccgcctccggcttcatcttctccagctacggaatgcactgggtccgacaggcccctggcaaaggattggaatgggtcgccgtgatttggtacgacggctccaacaagtactacgccgactccgtgaagggcagattcaccatctctcgggacaactccaagaacaccctgtacctgcagatgaactccctgagagccgaggacaccgccatgtactactgcgccagagatcactacggctccggcacctactacatcgactattggggccagggcaccctggtcacagtgtcctctgcttctaccaagggacccagcgtgttccctctggctccttccagcaagtctacctctggcggaacagctgctctgggctgcctggtcaaggactactttcctgagcctgtgaccgtgtcctggaactctggcgctctgacatctggcgtgcacacctttccagctgtgctgcagtcctccggcctgtactctctgtcctctgtcgtgaccgtgccttccagctctctgggaacccagacctacatctgcaatgtgaaccacaagccttccaacaccaaggtggacaagaaggtggaacccaagtcctgcgacaagacccacacctgtcctccatgtcctgctccagaactgctcggcggtccctccgttttcctgtttccacctaagcctaaggacaccctgatgatctctcggacccctgaagtgacatgcgtggtggtggatgtgtcccacgaggatcccgaagtgaagttcaattggtacgtggacggcgtggaagtgcacaacgccaagaccaagcctagagaggaacagtacaactccacctacagagtggtgtccgtgctgaccgtgctgcaccaggattggctgaacggcaaagagtacaagtgcaaggtgtccaacaaggccctgcctgctcctatcgaaaagaccatctccaaggctaagggccagcctcgggaacctcaggtttacacactgcctccatctcgggacgagctgaccaagaatcaggtgtccctgacctgcctcgtgaagggcttctacccttctgatatcgccgtggaatgggagtccaacggccagcctgagaacaactacaagacaacccctcctgtgctggactccgacggctcattcttcctgtactccaagctgacagtggataagtcccggtggcagcagggcaacgtgttctcttgttctgtgatgcacgaggccctgcacaaccactacacccagaagagtctgtctctgtcccctggcaagtga

SEQ ID NO: 10 - protein, 451 aa, Artificial Sequence
  Synthetic Construct
QVQLVESGGGVVQPGGSLRLSCAASGFIFSSYGMHWVRQAPGKGLEWVAVIWYDGSNKYYADSVKGRFTISRDNSKNTLYLQMNSLRAEDTAMYYCARDHYGSGTYYIDYWGQGTLVTVSSASTKGPSVFPLAPSSKSTSGGTAALGCLVKDYFPEPVTVSWNSGALTSGVHTFPAVLQSSGLYSLSSVVTVPSSSLGTQTYICNVNHKPSNTKVDKKVEPKSCDKTHTCPPCPAPELLGGPSVFLFPPKPKDTLMISRTPEVTCVVVDVSHEDPEVKFNWYVDGVEVHNAKTKPREEQYNSTYRVVSVLTVLHQDWLNGKEYKCKVSNKALPAPIEKTISKAKGQPREPQVYTLPPSRDELTKNQVSLTCLVKGFYPSDIAVEWESNGQPENNYKTTPPVLDSDGSFFLYSKLTVDKSRWQQGNVFSCSVMHEALHNHYTQKSLSLSPGK

SEQ ID NO: 11 - DNA, 642 bp, Artificial Sequence
  16B12.1_LC
  CDS (1)..(642)
gagattgtgatgacccagtctcctgccacactgtccgtgtctccaggcgagagagctaccctgtcttgcagagcttctcagaccgtgtcctccaacctggcctggtatcagcagaagcctggacaggctccccggctgttgatctatggcgcttctaccagagccaccggctttcccgctagattctccggctctggctctggcacagagtttaccctgaccatctccagcctgcagtccgaggatttcgccgtgtactactgccagcagtacaacaactggtggaccttcggccagggcaccaaggtggaaatcaagagaaccgtggccgctccttccgtgttcatcttcccaccttccgacgagcagctgaagtctggcaccgcttctgtcgtgtgcctgctgaacaacttctaccctcgggaagccaaggtgcagtggaaggtggacaatgccctgcagagcggcaactcccaagagtctgtgaccgagcaggactccaaggacagcacctacagcctgtcctccacactgaccctgtccaaggccgactacgagaagcacaaggtgtacgcctgcgaagtgacccatcagggcctgtctagccctgtgaccaagtctttcaaccggggcgagtgttga

SEQ ID NO: 12 - protein, 213 aa, Artificial Sequence
  Synthetic Construct
EIVMTQSPATLSVSPGERATLSCRASQTVSSNLAWYQQKPGQAPRLLIYGASTRATGFPARFSGSGSGTEFTLTISSLQSEDFAVYYCQQYNNWWTFGQGTKVEIKRTVAAPSVFIFPPSDEQLKSGTASVVCLLNNFYPREAKVQWKVDNALQSGNSQESVTEQDSKDSTYSLSSTLTLSKADYEKHKVYACEVTHQGLSSPVTKSFNRGEC

SEQ ID NO: 13 - DNA, 1461 bp, Artificial Sequence
  anti-CD3-scFv
  CDS (1)..(1461)
gaagtacagctggtggagtctggcggaggtcttatccagcccggaggttctctgcgcctgagctgtgcagcttccggtttcaccttcaacacctatgccatgaattgggtacgccaggctccaggaaaatgtctggagtgggtggctcggattcgaagcaaatacaacaattatgcaacctactatgccgacagtgtcaaggaccgcttcaccataagtcgggatgactccaagagcactctgtatctgcagatgaacaacttgagggccgaggataccgccgtttactattgcgtaaggcatggcaacttcggtaattcctacgtgtcctggtttgcctattggggccaagggacgctggttacagtgtcaagtggaaagcccgggtctggcaaacctgggagtggcaagcccgggagtgggaaaccaggatcccaggctgttgtcactcaagaacccagtctcactgtttctccaggcggtacagtcacactcacatgtcgtagcagcactggggctgtgaccaccagcaactatgcaaactgggtccagcagaaacccggtcaagctcccagaggattgattggcggtaccaataagcgggcccctgggactcctgctcgattttctggctccttgcttggagataaagccgcactgactttgagcggcgctcaaccagaggacgaagcagagtactattgtgctctgtggtactccaacctctgggtgtttggctgtggcaccaaggtaacagtgctggaacctaagtcaagcgacaaaacacacacctgtcctccctgtccagcaccagaggcagctggtggcccatctgtctttctgttcccaccaaagcccaaggacactctgatgatctcacgaacacccgaagtgacttgcgtagtggtggacgtttctcatgaggatccagaggtcaagttcaactggtacgtggatggagtggaagtgcacaatgccaaaacaaagccccgtgaggagcagtacggctccacgtacagggttgtctccgttttgaccgtcctgcatcaggattggcttaacggaaaagagtataagtgcaaggtatccaataaggcccttcccgcccctatcgagaaaactatcagcaaggccaaaggacagcccagagagccccaggtgtacactttgcctccttctagggatgaactcaccaagaatcaggttagcctgtggtgcctggtgaaggggttttacccatccgatattgccgtggagtgggaaagcaatggccaacccgagaacaactataagacaactcctcctgtgctggactcagatggaagtttcttcctgtacagcaagctcacagtggacaagagcagatggcagcagggcaatgtgttttcttgctctgtcatgcacgaagccctgcacaatcactacacccagaaatcccttagtctgtcacctgggaagtga

SEQ ID NO: 14 - protein, 486 aa, Artificial Sequence
  Synthetic Construct
EVQLVESGGGLIQPGGSLRLSCAASGFTFNTYAMNWVRQAPGKCLEWVARIRSKYNNYATYYADSVKDRFTISRDDSKSTLYLQMNNLRAEDTAVYYCVRHGNFGNSYVSWFAYWGQGTLVTVSSGKPGSGKPGSGKPGSGKPGSQAVVTQEPSLTVSPGGTVTLTCRSSTGAVTTSNYANWVQQKPGQAPRGLIGGTNKRAPGTPARFSGSLLGDKAALTLSGAQPEDEAEYYCALWYSNLWVFGCGTKVTVLEPKSSDKTHTCPPCPAPEAAGGPSVFLFPPKPKDTLMISRTPEVTCVVVDVSHEDPEVKFNWYVDGVEVHNAKTKPREEQYGSTYRVVSVLTVLHQDWLNGKEYKCKVSNKALPAPIEKTISKAKGQPREPQVYTLPPSRDELTKNQVSLWCLVKGFYPSDIAVEWESNGQPENNYKTTPPVLDSDGSFFLYSKLTVDKSRWQQGNVFSCSVMHEALHNHYTQKSLSLSPGK

SEQ ID NO: 15 - protein, 4 aa, Artificial Sequence
  GGGS linker
  PEPTIDE (1)..(4)
GGGS

SEQ ID NO: 16 - protein, 4 aa, Artificial Sequence
  SGGG linker
  PEPTIDE (1)..(4)
SGGG

SEQ ID NO: 17 - protein, 5 aa, Artificial Sequence
  GGGGS linker
  PEPTIDE (1)..(5)
GGGGS

SEQ ID NO: 18 - protein, 5 aa, Artificial Sequence
  SGGGG linker
  PEPTIDE (1)..(5)
SGGGG

SEQ ID NO: 19 - protein, 6 aa, Artificial Sequence
  GGGGGS linker
  PEPTIDE (1)..(6)
GGGGGS

SEQ ID NO: 20 - protein, 6 aa, Artificial Sequence
  SGGGGG linker
  PEPTIDE (1)..(6)
SGGGGG

SEQ ID NO: 21 - protein, 7 aa, Artificial Sequence
  GGGGGGS linker
  PEPTIDE (1)..(7)
GGGGGGS

SEQ ID NO: 22 - protein, 7 aa, Artificial Sequence
  SGGGGGG linker
  PEPTIDE (1)..(7)
SGGGGGG

SEQ ID NO: 23 - protein, 5 aa, Artificial Sequence
  GKPGS linker
  PEPTIDE (1)..(5)
GKPGS

SEQ ID NO: 24 - protein, 5 aa, Artificial Sequence
  16B11&16B12_HCDR1
  BINDING (1)..(5)
SYGMH

SEQ ID NO: 25 - protein, 17 aa, Artificial Sequence
  16B11_HCDR2
  BINDING (1)..(16)
VIWYDGRNKYYADSVKG

SEQ ID NO: 26 - protein, 17 aa, Artificial Sequence
  16B12_HCDR2
  BINDING (1)..(16)
VIWYDGSNKYYADSVKG

SEQ ID NO: 27 - protein, 12 aa, Artificial Sequence
  16B11_HCDR3
  BINDING (1)..(12)
DHSGSGSYYIDY

SEQ ID NO: 28 - protein, 12 aa, Artificial Sequence
  16B12_HCDR3
  BINDING (1)..(12)
DHYGSGTYYIDY

SEQ ID NO: 29 - protein, 11 aa, Artificial Sequence
  16B11_LCDR1
  BINDING (1)..(9)
RASQSVSSNLA

SEQ ID NO: 30 - protein, 11 aa, Artificial Sequence
  16B12_LCDR1
  BINDING (1)..(9)
RASQTVSSNLA

SEQ ID NO: 31 - protein, 7 aa, Artificial Sequence
  16B11&16B12_LCDR2
  BINDING (1)..(5)
GASTRAT

SEQ ID NO: 32 - protein, 8 aa, Artificial Sequence
  16B11_LCDR3
  BINDING (1)..(8)
QQYNNFWT

SEQ ID NO: 33 - protein, 8 aa, Artificial Sequence
  16B12_LCDR3
  BINDING (1)..(8)
QQYNNWWT

SEQ ID NO: 34 - protein, 121 aa, Artificial Sequence
  16B11_VH
  BINDING (1)..(114)
QVQLVESGGGVVQPGRSLRLSCAASGFTFSSYGMHWVRQAPGKGLEWVAVIWYDGRNKYYADSVKGRFTISRDNSKNTLYLQMNSLRAEDTAVYYCTRDHSGSGSYYIDYWGQGTLVTVSS

SEQ ID NO: 35 - protein, 121 aa, Artificial Sequence
  16B12_VH
  BINDING (1)..(113)
QVQLVESGGGVVQPGRSLRLSCAASGFIFSSYGMHWVRQAPGKGLEWVAVIWYDGSNKYYADSVKGRFTISRDNSKNTLYLQMNSLRAEDTAMYYCARDHYGSGTYYIDYWGQGTLVTVSS

SEQ ID NO: 36 - protein, 107 aa, Artificial Sequence
  16B11_VL
  BINDING (1)..(97)
EIAMTQSPATLSVSPGERATLSCRASQSVSSNLAWYQQKPGQAPRLLIYGASTRATGLPARFSGSGSGTEFTLTISSLQSEDFAVYYCQQYNNFWTFGQGTKVEIKR

SEQ ID NO: 37 - protein, 107 aa, Artificial Sequence
  16B12_VL
  BINDING (1)..(98)
EIVMTQSPATLSVSPGERATLSCRASQTVSSNLAWYQQKPGQAPRLLIYGASTRATGFPARFSGSGSGTEFTLTISSLQSEDFAVYYCQQYNNWWTFGQGTKVEIKR

SEQ ID NO: 38 - protein, 19 aa, Artificial Sequence
  signal sequence
  PEPTIDE (1)..(19)
MEWSWVFLFFLSVTTGVHS

SEQ ID NO: 39 - protein, 19 aa, Artificial Sequence
  signal sequence
  PEPTIDE (1)..(19)
MGWSCIILFLVATATGVHS

SEQ ID NO: 40 - protein, 19 aa, Artificial Sequence
  signal sequence
  PEPTIDE (1)..(19)
MEWSWVFLFFLSVTTGVHS

SEQ ID NO: 41 - protein, 30 aa, Artificial Sequence
  mouseTSPAN8 126-155
KLLSDNTDEAKDFQKAMIVFQSEFKCCGLE

SEQ ID NO: 42 - protein, 30 aa, Artificial Sequence
  ratTSPAN8 126-155
KLLSETSNEAKEVQKAMIAFQSEFKCCGLR

SEQ ID NO: 43 - protein, 30 aa, Artificial Sequence
  Macaca fascicula TSPAN8 126-155
KLLSTTGESAKQFQQAMAEFQKEFKCCGLV